European Patent Application EP 4 306 125 A1, published January 17, 2024. Title: Immunogenic personalised cancer vaccines. Applicant: Universiät Zürich. The sequence listing filed with the application follows.

SEQUENCE LISTING (175 sequences)

SEQ ID NO: 1 - protein, 9 aa, Homo sapiens
SPRVKWTFL

SEQ ID NO: 2 - protein, 9 aa, Homo sapiens
SPRLKWTFL

SEQ ID NO: 3 - protein, 9 aa, Homo sapiens
EMISVLGPI

SEQ ID NO: 4 - protein, 9 aa, Homo sapiens
EMISLLGPI

SEQ ID NO: 5 - protein, 9 aa, Homo sapiens
DLRKRRVLF

SEQ ID NO: 6 - protein, 9 aa, Homo sapiens
DLRQRRVLF

SEQ ID NO: 7 - protein, 9 aa, Homo sapiens
DLRNRRVLF

SEQ ID NO: 8 - protein, 9 aa, Homo sapiens
CTIDVYMIM

SEQ ID NO: 9 - protein, 9 aa, Homo sapiens
CTIDLYMIM

SEQ ID NO: 10 - protein, 9 aa, Homo sapiens
MPNQAQMRI

SEQ ID NO: 11 - protein, 9 aa, Homo sapiens
MPQQAQMRI

SEQ ID NO: 12 - protein, 9 aa, Homo sapiens
NIGCRFPYL

SEQ ID NO: 13 - protein, 9 aa, Homo sapiens
NIGCKFPYL

SEQ ID NO: 14 - protein, 9 aa, Homo sapiens
MPKKKRLSA

SEQ ID NO: 15 - protein, 9 aa, Homo sapiens
MPKQKRLSA

SEQ ID NO: 16 - protein, 9 aa, Homo sapiens
MPKAKRLSA

SEQ ID NO: 17 - protein, 9 aa, Homo sapiens
VVVANVSKY

SEQ ID NO: 18 - protein, 9 aa, Homo sapiens
VVVAQVSKY

SEQ ID NO: 19 - protein, 9 aa, Homo sapiens
HTIKDFWRM

SEQ ID NO: 20 - protein, 9 aa, Homo sapiens
HTIKEFWRM

SEQ ID NO: 21 - protein, 9 aa, Homo sapiens
TMIEKFAVL

SEQ ID NO: 22 - protein, 9 aa, Homo sapiens
TMIQKFAVL

SEQ ID NO: 23 - protein, 9 aa, Homo sapiens
TMIDKFAVL

SEQ ID NO: 24 - protein, 9 aa, Homo sapiens
TTIGLLYPF

SEQ ID NO: 25 - protein, 9 aa, Homo sapiens
TTIGILYPF

SEQ ID NO: 26 - protein, 9 aa, Homo sapiens
LLRNRLQAL

SEQ ID NO: 27 - protein, 9 aa, Homo sapiens
LLRQRLQAL

SEQ ID NO: 28 - protein, 9 aa, Homo sapiens
FLRYRPLIL

SEQ ID NO: 29 - protein, 9 aa, Homo sapiens
FLRWRPLIL

SEQ ID NO: 30 - protein, 9 aa, Homo sapiens
FLRRKAEAM

SEQ ID NO: 31 - protein, 9 aa, Homo sapiens
FLRKKAEAM

SEQ ID NO: 32 - protein, 9 aa, Homo sapiens
TVIEDMLAM

SEQ ID NO: 33 - protein, 9 aa, Homo sapiens
TVIEEMLAM

SEQ ID NO: 34 - protein, 9 aa, Homo sapiens
MPRDILIVV

SEQ ID NO: 35 - protein, 9 aa, Homo sapiens
MPKDILIVV

SEQ ID NO: 36 - protein, 9 aa, Homo sapiens
MPFRLKDPV

SEQ ID NO: 37 - protein, 9 aa, Homo sapiens
MPYRLKDPV

SEQ ID NO: 38 - protein, 9 aa, Homo sapiens
FPRARTVSV

SEQ ID NO: 39 - protein, 9 aa, Homo sapiens
FPRSRTVSV

SEQ ID NO: 40 - protein, 9 aa, Homo sapiens
MPISSVRFV

SEQ ID NO: 41 - protein, 9 aa, Homo sapiens
MPLSSVRFV

SEQ ID NO: 42 - protein, 9 aa, Homo sapiens
TSINNMAAF

SEQ ID NO: 43 - protein, 9 aa, Homo sapiens
TSINQMAAF

SEQ ID NO: 44 - protein, 9 aa, Homo sapiens
HTIEDFWRM

SEQ ID NO: 45 - protein, 9 aa, Homo sapiens
HTIEEFWRM

SEQ ID NO: 46 - protein, 9 aa, Homo sapiens
MAFANSPWV

SEQ ID NO: 47 - protein, 9 aa, Homo sapiens
MAMANSPWV

SEQ ID NO: 48 - protein, 9 aa, Homo sapiens
MPYTSMPMM

SEQ ID NO: 49 - protein, 9 aa, Homo sapiens
MPFTSMPMM

SEQ ID NO: 50 - protein, 9 aa, Homo sapiens
EIIQPLLDM

SEQ ID NO: 51 - protein, 9 aa, Homo sapiens
EIIQPLIDM

SEQ ID NO: 52 - protein, 9 aa, Homo sapiens
DVISNIETF

SEQ ID NO: 53 - protein, 9 aa, Homo sapiens
DVISQIETF

SEQ ID NO: 54 - protein, 9 aa, Homo sapiens
FMRKRIEAI

SEQ ID NO: 55 - protein, 9 aa, Homo sapiens
FMRQRIEAI

SEQ ID NO: 56 - protein, 9 aa, Homo sapiens
HAIHYVNKI

SEQ ID NO: 57 - protein, 9 aa, Homo sapiens
HAIHFVNKI

SEQ ID NO: 58 - protein, 9 aa, Homo sapiens
LPKGFLASL

SEQ ID NO: 59 - protein, 9 aa, Homo sapiens
LPKPFLASL

SEQ ID NO: 60 - protein, 9 aa, Homo sapiens
LPKAFLASL

SEQ ID NO: 61 - protein, 9 aa, Homo sapiens
AARARLHPL

SEQ ID NO: 62 - protein, 9 aa, Homo sapiens
AARSRLHPL

SEQ ID NO: 63 - protein, 9 aa, Homo sapiens
LRRLHGTTL

SEQ ID NO: 64 - protein, 9 aa, Homo sapiens
LRRIHGTTL

SEQ ID NO: 65 - protein, 9 aa, Homo sapiens
IMRGRGRGV

SEQ ID NO: 66 - protein, 9 aa, Homo sapiens
IMRPRGRGV

SEQ ID NO: 67 - protein, 9 aa, Homo sapiens
IMRARGRGV

SEQ ID NO: 68 - protein, 12 aa, Homo sapiens
KFFLSDEFNIAT

SEQ ID NO: 69 - protein, 12 aa, Homo sapiens
KFFLSEEFNIAT

SEQ ID NO: 70 - protein, 13 aa, Homo sapiens
AAIRNDVAKQRAA

SEQ ID NO: 71 - protein, 13 aa, Homo sapiens
AAIRNDLAKQRAA

SEQ ID NO: 72 - protein, 13 aa, Homo sapiens
TLMIQNAGAVSAV

SEQ ID NO: 73 - protein, 13 aa, Homo sapiens
TLMIQNSGAVSAV

SEQ ID NO: 74 - protein, 13 aa, Homo sapiens
LRYEVDTVLRYEV

SEQ ID NO: 75 - protein, 13 aa, Homo sapiens
LRYEVDSVLRYEV

SEQ ID NO: 76 - protein, 11 aa, Homo sapiens
FFFDIDLLLQR

SEQ ID NO: 77 - protein, 11 aa, Homo sapiens
FFFDIELLLQR

SEQ ID NO: 78 - protein, 11 aa, Homo sapiens
NDIYRIFAELE

SEQ ID NO: 79 - protein, 11 aa, Homo sapiens
NDIYRIYAELE

SEQ ID NO: 80 - protein, 11 aa, Homo sapiens
NDIYKIFAELE

SEQ ID NO: 81 - protein, 13 aa, Homo sapiens
LKMLNIPSINVHH

SEQ ID NO: 82 - protein, 13 aa, Homo sapiens
LKMLHIPSINVHH

SEQ ID NO: 83 - protein, 13 aa, Homo sapiens
LKMLQIPSINVHH

SEQ ID NO: 84 - protein, 13 aa, Homo sapiens
SIYVYALPLKMLN

SEQ ID NO: 85 - protein, 13 aa, Homo sapiens
SIYVYAVPLKMLN

SEQ ID NO: 86 - protein, 13 aa, Homo sapiens
APLEGVLVELEVL

SEQ ID NO: 87 - protein, 13 aa, Homo sapiens
APLEGVIVELEVL

SEQ ID NO: 88 - protein, 13 aa, Homo sapiens
APLEAVLVELEVL

SEQ ID NO: 89 - protein, 13 aa, Homo sapiens
GSLTLAPPLLRVS

SEQ ID NO: 90 - protein, 13 aa, Homo sapiens
GSLTLTPPLLRVS

SEQ ID NO: 91 - protein, 12 aa, Homo sapiens
VLLAFLQYRRLR

SEQ ID NO: 92 - protein, 12 aa, Homo sapiens
VLLTFLQYRRLR

SEQ ID NO: 93 - protein, 13 aa, Homo sapiens
NRLLYNATTNILE

SEQ ID NO: 94 - protein, 13 aa, Homo sapiens
NRLLYNSTTNILE

SEQ ID NO: 95 - protein, 13 aa, Homo sapiens
FGSLAFLPESFDG

SEQ ID NO: 96 - protein, 13 aa, Homo sapiens
FGSLAFIPESFDG

SEQ ID NO: 97 - protein, 13 aa, Homo sapiens
FGSLSFLPESFDG

SEQ ID NO: 98 - protein, 13 aa, Homo sapiens
GRILHNGAYSLTL

SEQ ID NO: 99 - protein, 13 aa, Homo sapiens
GRILHNPAYSLTL

SEQ ID NO: 100 - protein, 13 aa, Homo sapiens
GRILHNAAYSLTL

SEQ ID NO: 101 - protein, 13 aa, Homo sapiens
MSYLEDVRLVHRD

SEQ ID NO: 102 - protein, 13 aa, Homo sapiens
MSYLEDLRLVHRD

SEQ ID NO: 103 - protein, 13 aa, Homo sapiens
RLVHRDLAARNVL

SEQ ID NO: 104 - protein, 13 aa, Homo sapiens
RLVHRDIAARNVL

SEQ ID NO: 105 - protein, 13 aa, Homo sapiens
LPFFLLPSFFNNT

SEQ ID NO: 106 - protein, 13 aa, Homo sapiens
LPFFLLASFFNNT

SEQ ID NO: 107 - protein, 13 aa, Homo sapiens
PSFFNNTSLARFF

SEQ ID NO: 108 - protein, 13 aa, Homo sapiens
PSFFNNSSLARFF

SEQ ID NO: 109 - protein, 12 aa, Homo sapiens
SSYFTFQLQNIV

SEQ ID NO: 110 - protein, 12 aa, Homo sapiens
SSYFTFNLQNIV

SEQ ID NO: 111 - protein, 13 aa, Homo sapiens
TKFIHTKPNRFEE

SEQ ID NO: 112 - protein, 13 aa, Homo sapiens
TKFIHTRPNRFEE

SEQ ID NO: 113 - protein, 13 aa, Homo sapiens
VCVMLNSNVLLWL

SEQ ID NO: 114 - protein, 13 aa, Homo sapiens
VCVMLNTNVLLWL

SEQ ID NO: 115 - protein, 13 aa, Homo sapiens
NAFVNVLAEPPRI

SEQ ID NO: 116 - protein, 13 aa, Homo sapiens
NAFVNVIAEPPRI

SEQ ID NO: 117 - protein, 13 aa, Homo sapiens
NAFVQVLAEPPRI

SEQ ID NO: 118 - protein, 13 aa, Homo sapiens
ASFSSELFRHLHT

SEQ ID NO: 119 - protein, 13 aa, Homo sapiens
ASFSTELFRHLHT

SEQ ID NO: 120 - protein, 13 aa, Homo sapiens
HLIVSNSASSENM

SEQ ID NO: 121 - protein, 13 aa, Homo sapiens
HLIVSNTASSENM

SEQ ID NO: 122 - protein, 13 aa, Homo sapiens
KHIRSQRNYLVQT

SEQ ID NO: 123 - protein, 13 aa, Homo sapiens
KHIRSQKNYLVQT

SEQ ID NO: 124 - protein, 13 aa, Homo sapiens
RAEIVTEAEPEVD

SEQ ID NO: 125 - protein, 13 aa, Homo sapiens
RAEIVTDAEPEVD

SEQ ID NO: 126 - protein, 13 aa, Homo sapiens
RAEIVSEAEPEVD

SEQ ID NO: 127 - protein, 13 aa, Homo sapiens
KTFDWTQFRIISR

SEQ ID NO: 128 - protein, 13 aa, Homo sapiens
KTFDWTNFRIISR

SEQ ID NO: 129 - protein, 13 aa, Homo sapiens
NKFLSEIEDELFN

SEQ ID NO: 130 - protein, 13 aa, Homo sapiens
NKFLAEIEDELFN

SEQ ID NO: 131 - protein, 13 aa, Homo sapiens
VAAFAYQIEELMI

SEQ ID NO: 132 - protein, 13 aa, Homo sapiens
VAAFAYNIEELMI

SEQ ID NO: 133 - protein, 13 aa, Homo sapiens
VAAFSYQIEELMI

SEQ ID NO: 134 - protein, 12 aa, Homo sapiens
LFFEFYRLLHDA

SEQ ID NO: 135 - protein, 12 aa, Homo sapiens
LFFDFYRLLHDA

SEQ ID NO: 136 - protein, 11 aa, Homo sapiens
FKIQYLQFLAY

SEQ ID NO: 137 - protein, 11 aa, Homo sapiens
FKIQYLNFLAY

SEQ ID NO: 138 - protein, 13 aa, Homo sapiens
REFTKATNVRLRF

SEQ ID NO: 139 - protein, 13 aa, Homo sapiens
REFTKASNVRLRF

SEQ ID NO: 140 - protein, 13 aa, Homo sapiens
GSFLRIPSLHLLL

SEQ ID NO: 141 - protein, 13 aa, Homo sapiens
GSFLKIPSLHLLL

SEQ ID NO: 142 - protein, 13 aa, Homo sapiens
HPFALTLFEDILY

SEQ ID NO: 143 - protein, 13 aa, Homo sapiens
HPFALSLFEDILY

SEQ ID NO: 144 - protein, 11 aa, Homo sapiens
LEFAQFPFLLR

SEQ ID NO: 145 - protein, 11 aa, Homo sapiens
LEFANFPFLLR

SEQ ID NO: 146 - protein, 13 aa, Homo sapiens
DVFQTVKSLRLQR

SEQ ID NO: 147 - protein, 13 aa, Homo sapiens
DVFQSVKSLRLQR

SEQ ID NO: 148 - protein, 12 aa, Homo sapiens
LQFLADLEELIT

SEQ ID NO: 149 - protein, 12 aa, Homo sapiens
LQFLSDLEELIT

SEQ ID NO: 150 - protein, 13 aa, Homo sapiens
LQFLADLEELITK

SEQ ID NO: 151 - protein, 13 aa, Homo sapiens
LQFLSDLEELITK

SEQ ID NO: 152 - protein, 13 aa, Homo sapiens
MGFIQAMSALRGM

SEQ ID NO: 153 - protein, 13 aa, Homo sapiens
MGFIQSMSALRGM

SEQ ID NO: 154 - protein, 11 aa, Homo sapiens
PALEAHCVEFL

SEQ ID NO: 155 - protein, 11 aa, Homo sapiens
PALEAHSVEFL

SEQ ID NO: 156 - protein, 13 aa, Homo sapiens
WLVLGFLWPLLTL

SEQ ID NO: 157 - protein, 13 aa, Homo sapiens
WLVLPFLWPLLTL

SEQ ID NO: 158 - protein, 12 aa, Homo sapiens
FRLKINEETPLK

SEQ ID NO: 159 - protein, 12 aa, Homo sapiens
FRLKINEGTPLK

SEQ ID NO: 160 - protein, 12 aa, Homo sapiens
FRLKINQGTPLK

SEQ ID NO: 161 - protein, 12 aa, Homo sapiens
FRLKINDGTPLK

SEQ ID NO: 162 - protein, 13 aa, Homo sapiens
TGINFDNPSVQKA

SEQ ID NO: 163 - protein, 13 aa, Homo sapiens
TGINFDEPSVQKA

SEQ ID NO: 164 - protein, 13 aa, Homo sapiens
TGINFDQPSVQKA

SEQ ID NO: 165 - protein, 13 aa, Homo sapiens
LQFVKDHPLMDDL

SEQ ID NO: 166 - protein, 13 aa, Homo sapiens
LQFVKDQPLMDDL

SEQ ID NO: 167 - protein, 13 aa, Homo sapiens
LQFVKDKPLMDDL

SEQ ID NO: 168 - protein, 13 aa, Homo sapiens
QPVEFNHAINYVN

SEQ ID NO: 169 - protein, 13 aa, Homo sapiens
QPVEFNHAIHYVN

SEQ ID NO: 170 - protein, 13 aa, Homo sapiens
QPVEFNQAINYVN

SEQ ID NO: 171 - protein, 13 aa, Homo sapiens
QPVEFNKAINYVN

SEQ ID NO: 172 - protein, 13 aa, Homo sapiens
RQLQVDRTKLSRA

SEQ ID NO: 173 - protein, 13 aa, Homo sapiens
RQLQVDKTKLSRA

SEQ ID NO: 174 - protein, 12 aa, Homo sapiens
PILSADDLLGSP

SEQ ID NO: 175 - protein, 12 aa, Homo sapiens
PILSADELLGSP